European Patent Application EP 4 269 624 A1, published November 1, 2023. Title: DPC细胞鉴定分类用标记物基因、筛选方法及应用. Applicant: 武汉睿健医药科技有限公司. The sequence listing filed with the application follows.

SEQUENCE LISTING (24 sequences)

SEQ ID NO: 1 - DNA, 24 bp, Artificial Sequence
gcagcagcaacacaatgttattcg

SEQ ID NO: 2 - DNA, 23 bp, Artificial Sequence
tggcattctctttggctcagacc

SEQ ID NO: 3 - DNA, 21 bp, Artificial Sequence
gctgctgctctgccagttcat

SEQ ID NO: 4 - DNA, 24 bp, Artificial Sequence
tgtgttgtcattcacgtcctcctc

SEQ ID NO: 5 - DNA, 22 bp, Artificial Sequence
acatcaacagcgagcacatcca

SEQ ID NO: 6 - DNA, 22 bp, Artificial Sequence
cgaggcgtgagtatgacttccg

SEQ ID NO: 7 - DNA, 24 bp, Artificial Sequence
ccatgtcattgaccgtgtgcttac

SEQ ID NO: 8 - DNA, 24 bp, Artificial Sequence
gcctccaatatgtccgatgtgatg

SEQ ID NO: 9 - DNA, 21 bp, Artificial Sequence
ttcacagcagcaggcgtcttg

SEQ ID NO: 10 - DNA, 23 bp, Artificial Sequence
cacagccaggaagagcacatcac

SEQ ID NO: 11 - DNA, 23 bp, Artificial Sequence
tccactgtgagacaagcggttac

SEQ ID NO: 12 - DNA, 24 bp, Artificial Sequence
tcctccatcggtagagtagtccaa

SEQ ID NO: 13 - DNA, 24 bp, Artificial Sequence
aacagtgaccattacgtgccagta

SEQ ID NO: 14 - DNA, 23 bp, Artificial Sequence
ccacaatcagcaagcatccatcc

SEQ ID NO: 15 - DNA, 23 bp, Artificial Sequence
tggttgatgccactgccatgatc

SEQ ID NO: 16 - DNA, 24 bp, Artificial Sequence
agtctaagagcccacccaacaagg

SEQ ID NO: 17 - DNA, 24 bp, Artificial Sequence
tgacagtggcatcagagtgaagag

SEQ ID NO: 18 - DNA, 24 bp, Artificial Sequence
aaggtccagaatgagtggcaagaa

SEQ ID NO: 19 - DNA, 22 bp, Artificial Sequence
aggaggcagtggacatcgtagg

SEQ ID NO: 20 - DNA, 24 bp, Artificial Sequence
cagagcaggaggttggaacagaac

SEQ ID NO: 21 - DNA, 24 bp, Artificial Sequence
tcctggtcaatctgtggtactcct

SEQ ID NO: 22 - DNA, 24 bp, Artificial Sequence
ctggcttgatgtctctgtggatga

SEQ ID NO: 23 - DNA, 24 bp, Artificial Sequence
cctggagaggaactgagtgtcacc

SEQ ID NO: 24 - DNA, 24 bp, Artificial Sequence
gcagactgagggagatccgagaag